European Patent Application EP 4 501 964 A1, published February 5, 2025. Title: HLA-G SPECIFIC ANTIBODIES AND USEDS THEREOF. Applicant: 에이치케이이노엔. The sequence listing filed with the application follows.

SEQUENCE LISTING (44 sequences)

SEQ ID NO: 1 - protein, 5 aa, Artificial Sequence
DYAMS

SEQ ID NO: 2 - protein, 17 aa, Artificial Sequence
VISHDGDRVYYADSVKG

SEQ ID NO: 3 - protein, 12 aa, Artificial Sequence
GPRRIANAIFDY

SEQ ID NO: 4 - protein, 121 aa, Artificial Sequence
EVQLLESGGGLVQPGGSLRLSCAASGFTFSDYAMSWVRQAPGKGLEWVSVISHDGDRVYYADSVKGRFTISRDNSKNTLYLQMNSLRAEDTAVYYCAKGPRRIANAIFDYWGQGTLVTVSS

SEQ ID NO: 5 - protein, 13 aa, Artificial Sequence
SGSSSNIGHSYVS

SEQ ID NO: 6 - protein, 7 aa, Artificial Sequence
GDNNRPS

SEQ ID NO: 7 - protein, 11 aa, Artificial Sequence
QSYDSSLSGYV

SEQ ID NO: 8 - protein, 110 aa, Artificial Sequence
QLVLTQPPSVSGAPGQKVTISCSGSSSNIGHSYVSWYQQLPGTAPKLLIYGDNNRPSGVPDRFSGSKSGTSASLAITGLQAEDEADYYCQSYDSSLSGYVFGTGTKVTVL

SEQ ID NO: 9 - protein, 5 aa, Artificial Sequence
DYAMS

SEQ ID NO: 10 - protein, 17 aa, Artificial Sequence
VISHDGGSIYYADSVKG

SEQ ID NO: 11 - protein, 12 aa, Artificial Sequence
GPRRIANAIFDY

SEQ ID NO: 12 - protein, 121 aa, Artificial Sequence
EVQLLESGGGLVQPGGSLRLSCAASGFTFSDYAMSWVRQAPGKGLEWVSVISHDGGSIYYADSVKGRFTISRDNSKNTLYLQMNSLRAEDTAVYYCAKGPRRIANAIFDYWGQGTLVTVSS

SEQ ID NO: 13 - protein, 13 aa, Artificial Sequence
SGSNSNIGNSYVS

SEQ ID NO: 14 - protein, 7 aa, Artificial Sequence
GSTNRPS

SEQ ID NO: 15 - protein, 11 aa, Artificial Sequence
QSYDSSLSGYV

SEQ ID NO: 16 - protein, 110 aa, Artificial Sequence
QFVLTQPPSVSAAPGQKVTISCSGSNSNIGNSYVSWYQQVPGAAPRLLIYGSTNRPSGVPDRFSGSKSGTSASLAITGLQAEDEADYYCQSYDSSLSGYVFGTGTKVTVL

SEQ ID NO: 17 - protein, 5 aa, Artificial Sequence
DYSMS

SEQ ID NO: 18 - protein, 17 aa, Artificial Sequence
AISPDRSLEYYADSVKG

SEQ ID NO: 19 - protein, 12 aa, Artificial Sequence
GPRHLTNNIFDY

SEQ ID NO: 20 - protein, 121 aa, Artificial Sequence
EVQLLESGGGLVQPGGSLRLSCAASGFTFSDYSMSWVRQAPGKGLEWVSAISPDRSLEYYADSVKGRFTISRDNSKNTLYLQMNSLRAEDTAVYYCAKGPRHLTNNIFDYWGQGTLVTVSS

SEQ ID NO: 21 - protein, 13 aa, Artificial Sequence
SGSSSNIGHSYVS

SEQ ID NO: 22 - protein, 7 aa, Artificial Sequence
GNIHRPS

SEQ ID NO: 23 - protein, 11 aa, Artificial Sequence
GVWDSSLSAVV

SEQ ID NO: 24 - protein, 110 aa, Artificial Sequence
QFVLTQPPSVSAAPGQKVTISCSGSSSNIGHSYVSWYQQLPGTAPKLLIYGNIHRPSGVPDRFSGSTSGTSASLAITGLQADDEADYYCGVWDSSLSAVVFGGGTKLTVL

SEQ ID NO: 25 - protein, 5 aa, Artificial Sequence
DYSMS

SEQ ID NO: 26 - protein, 17 aa, Artificial Sequence
AISPDSGSKYYADSVKG

SEQ ID NO: 27 - protein, 12 aa, Artificial Sequence
GPRHLTNNIFDY

SEQ ID NO: 28 - protein, 121 aa, Artificial Sequence
EVQLLESGGGLVQPGGSLRLSCAASGFTFSDYSMSWVRQAPGKGLEWVSAISPDSGSKYYADSVKGRFTISRDNSKNTLYLQMNSLRAEDTAVYYCAKGPRHLTNNIFDYWGQGTLVTVSS

SEQ ID NO: 29 - protein, 13 aa, Artificial Sequence
TGSSSNIGSNYVS

SEQ ID NO: 30 - protein, 7 aa, Artificial Sequence
ADSNRPS

SEQ ID NO: 31 - protein, 11 aa, Artificial Sequence
ASWDYSLSGYV

SEQ ID NO: 32 - protein, 110 aa, Artificial Sequence
QSVLTQPPSASGTPGQRVTISCTGSSSNIGSNYVSWYQQLPGTAPKLLIYADSNRPSGVPDRFSGSKSGTSASLAISGLRSEDEADYYCASWDYSLSGYVFGGGTKLTVL

SEQ ID NO: 33 - protein, 460 aa, Artificial Sequence
MSRSVALAVLALLSLSGLEARIIPRHLQLGCGGSGGGGSGGGGSIQRTPKIQVYSRHPAENGKSNFLNCYVSGFHPSDIEVDLLKNGERIEKVEHSDLSFSKDWSFYLLYYTEFTPTEKDEYACRVNHVTLSQPKIVKWDRDMGGGGSGGGGSGGGGSGGGGSGSHSMRYFSAAVSRPGRGEPRFIAMGYVDDTQFVRFDSDSACPRMEPRAPWVEQEGPEYWEEETRNTKAHAQTDRMNLQTLRGCYNQSEASSHTLQWMIGCDLGSDGRLLRGYEQYAYDGKDYLALNEDLRSWTAADTAAQISKRKCEAANVAEQRRAYLEGTCVEWLHRYLENGKEMLQRADPPKTHVTHHPVFDYEATLRCWALGFYPAEIILTWQRDGEDQTQDVELVETRPAGDGTFQKWAAVVVPSGEEQRYTCHVQHEGLPEPLMLRWGSGLNDIFEAQKIEWHEHHHHHH

SEQ ID NO: 34 - protein, 6 aa, Homo sapiens
DYEATL

SEQ ID NO: 35 - protein, 13 aa, Homo sapiens
VVVPSGEEQRYTC

SEQ ID NO: 36 - protein, 16 aa, Homo sapiens
QRADPPKTHVTHHPVF

SEQ ID NO: 37 - DNA, 363 bp, Artificial Sequence
  source 1..363: mol_type = other DNA
gaggtgcagctgttggagtctgggggaggcttggtacagcctggggggtccctgagactctcctgtgcagcctctggattcacctttagcgattatgctatgagctgggtccgccaggctccagggaaggggctggagtgggtctcagtgatctctcatgatggcgatagagtatattacgctgattctgtaaaaggtcggttcaccatctccagagacaattccaagaacacgctgtatctgcaaatgaacagcctgagggccgaggacacggccgtgtattactgtgcgaaaggtcctaggcgtattgcgaatgcgattttcgactactggggccagggtacactggtcaccgtgagctca

SEQ ID NO: 38 - DNA, 330 bp, Artificial Sequence
  source 1..330: mol_type = other DNA
cagctcgtgctgactcagccgccctcagtgtctggggccccaggacagaaggtcaccatctcctgctctggaagcagctccaacattggacattcttatgtctcctggtaccagcaactcccaggaacagcccccaaactcctcatttatggtgacaacaatcggccctcaggggtccctgaccgattctctggctccaagtctggcacttcagcctccctggccatcactgggctccaggctgaggatgaggctgattattactgccagtcctatgacagcagcctgagtggttatgtcttcggaactgggaccaaggtcaccgtccta

SEQ ID NO: 39 - DNA, 363 bp, Artificial Sequence
  source 1..363: mol_type = other DNA
gaggtgcagctgttggagtctgggggaggcttggtacagcctggggggtccctgagactctcctgtgcagcctctggattcacctttagcgattatgctatgagctgggtccgccaggctccagggaaggggctggagtgggtctcagtgatctctcatgatggtggtagtatatattacgctgattctgtaaaaggtcggttcaccatctccagagacaattccaagaacacgctgtatctgcaaatgaacagcctgagggccgaggacacggccgtgtattactgtgcgaaaggtcctaggcgtattgcgaatgcgattttcgactactggggccagggtacactggtcaccgtgagctca

SEQ ID NO: 40 - DNA, 330 bp, Artificial Sequence
  source 1..330: mol_type = other DNA
cagttcgtgctgactcagccgccctcagtgtctgcggccccaggacagaaggtcaccatctcctgctctggaagcaactccaacattgggaacagttatgtctcctggtatcagcaagtcccaggagcagcccccagacttctcatctatggtagcaccaatcgcccttcaggagtccctgaccgattctctggctccaagtctggcacctcagcctccctggccatcactgggctccaggctgaggatgaggctgattattactgccagtcctatgacagcagcctgagtggttatgtcttcggaactgggaccaaggtcaccgtccta

SEQ ID NO: 41 - DNA, 363 bp, Artificial Sequence
  source 1..363: mol_type = other DNA
gaggtgcagctgttggagtctgggggaggcttggtacagcctggggggtccctaagactctcctgtgcagcctctggattcacctttagcgattattctatgagctgggtccgccaggctccagggaaggggctggagtgggtctcagcgatctctcctgatcgaagcttggaatattacgctgattctgtaaaaggtcggttcaccatctccagagacaattccaagaacacgctgtatctgcaaatgaacagcctgagagccgaggacacggccgtgtattactgtgcgaaaggtcctcgtcatctgacgaataatattttcgactactggggccagggtacactggtcaccgtgagctca

SEQ ID NO: 42 - DNA, 330 bp, Artificial Sequence
  source 1..330: mol_type = other DNA
cagttcgtgctgactcagccgccctcagtgtctgcggccccaggacagaaggtcaccatctcctgctctggaagcagctccaacattggacattcttatgtctcctggtaccagcaactcccaggaacagcccccaaactcctcatctatggaaacatccatcgcccctcaggggtccctgaccgattctctggctccacgtctggcacctcagcctccctggccatcactggactccaggccgatgatgaggctgattattattgcggagtatgggatagcagcctgagtgctgtggtattcggcggagggaccaagctgaccgtccta

SEQ ID NO: 43 - DNA, 363 bp, Artificial Sequence
  source 1..363: mol_type = other DNA
gaggtgcagctgttggagtctgggggaggcttggtacagcctggggggtccctaagactctcctgtgcagcctctggattcacctttagcgattattctatgagctgggtccgccaggctccagggaaggggctggagtgggtctcagcgatctctcctgatagtggtagtaaatattacgctgattctgtaaaaggtcggttcaccatctccagagacaattccaagaacacgctgtatctgcaaatgaacagcctgagagccgaggacacggccgtgtattactgtgcgaaaggtcctcgtcatctgacgaataatattttcgactactggggccagggtacactggtcaccgtgagctca

SEQ ID NO: 44 - DNA, 330 bp, Artificial Sequence
  source 1..330: mol_type = other DNA
cagtctgtgctgactcagccaccctcagcgtctgggacccccgggcagagggtcaccatctcttgtactggctcttcatctaatattggcagtaattatgtcagctggtaccagcagctcccaggaacggcccccaaactcctcatctatgctgatagtaatcggccaagcggggtccctgaccgattctctggctccaagtctggcacctcagcctccctggccatcagtgggctccggtccgaggatgaggctgattattactgtgcttcttgggattatagcctgagtggttatgtcttcggcggaggcaccaagctgacggtccta